European Patent Specification EP 3 749 680 B1, published April 3, 2024. Title: LIPID PRODUCTION. Applicant: Evonik Degussa GmbH. The sequence listing filed with the application follows.

SEQUENCE LISTING (21 sequences)

SEQ ID NO: 1 - DNA, 840 bp, Serratia rubidaea ATCC 27593
  rbwA (1)..(840)
atgaaaccagaaacagaaattgttcgcgtcggtgactggcaggtctatgtagagcgatatatttatccaggcgtcacggattccgtcatttgcgttaatggatctttttcaaccacgctggcttttcgcagctgcgtacgtaacttcaagaaccgggttaacgtcattctcttcgatctgccgttcctcggtcagtcccgtgagcataatgatttaaccaaaccgctgtcgaaaaccgatgaggttttcattctgcagagtttgattaaccattatgaaccgtcttatctgctctccatctcctggggcggactggcagcattgatggcgctctcctcccgccctcgctccatccgcaaagccgtggtggcctcgttctccaccaaggtgaacgacgcgatgaattactacgtcagtcagggcaagaaattactggatgaaggcaaaggcgatgaagcggcgatgctgctcaataccgaggttggcaaatatctgccgaatctgttgaagcaggtgaactacgaacacttgagacagtttgacgaatcagcgcaaaaacaggtgcgttaccacgtcgcgcaaattaccgaatttaatcaggcggactatatcgataccttccggcaaatcgatacgccgatactgttcatcaacggcgagcaggacgaatacactacagcgcaagatattaaggaactcagtaactatatcaataactgcgaatttattaccgtaccgcaggctggccactttatttatatggaaagccgctttgcggccgattatttcaacgacgtgatgaacggttttctgtttgttgaagaagcgatggcctcctga

SEQ ID NO: 2 - protein, 279 aa, Serratia rubidaea
  RbwA, 3-(3-hydroxyalkanoyloxy)alkanoic acids (HAAs) synthase (1)..(279)
MKPETEIVRVGDWQVYVERYIYPGVTDSVICVNGSFSTTLAFRSCVRNFKNRVNVILFDLPFLGQSREHNDLTKPLSKTDEVFILQSLINHYEPSYLLSISWGGLAALMALSSRPRSIRKAVVASFSTKVNDAMNYYVSQGKKLLDEGKGDEAAMLLNTEVGKYLPNLLKQVNYEHLRQFDESAQKQVRYHVAQITEFNQADYIDTFRQIDTPILFINGEQDEYTTAQDIKELSNYINNCEFITVPQAGHFIYMESRFAADYFNDVMNGFLFVEEAMAS

SEQ ID NO: 3 - DNA, 1176 bp, Serratia rubidaea ATCC 27593
  rbwB (1)..(1176)
atgagagtgataatatgcgccctggggtcctctggcgatgtttacccatgcatcgaaattggcgcgatattaaaagaaagaaaccatgatgtgcatatacttaccaatgaatacttcaaagattacgttgagtctcgcaatctttccttttcagcagtaggcagtaaagaggactttatccgttcagtacgtgacagccagctatgggagaagaaaacctcattaataaaaatatctgcatacatggctaattatcaggttggtatgtttcattcaatcgagaggttggtaaatgataattgtgtaattattcattctctttgggtattctcagccaaggtggttagcgaaaaatattcgttaaaacgattcccgataagccttaccaacgccaaccttaaactctgcccggggaaatttattagctggttggaaagaaagctcggcacctcattgaacctgaaggctgaactctttagacgccgcctggtttctccgctgttacaggaggtcatcgcctcgataagaaaatcagagaacctcccagccgataaaaacatctataccgacctggtagataggcgcttgaatcctattattttgtatgagccttggttctacgaaaaaaaaccgcagcacggattttatatggggttcctgttaaataaaaaccggacattagaccacgctccgataatcaaccgctttgtggacaaaaaaacggtggttttcttcaccagttgggcattgtctgatgaagcaggcataaatcatgtcttaagcagtctgaaagatgaaggtttgaaatgtgtactggtcacccccaccctcgacagcatccacgttgaagaaaatgtcatcagaacaccttaccttaatatggatagcatcaaaggatgtctgtttgccattcaccacggcggcatcggcaccagtgcccaactgcttaaaaacggcatacctcagttaatctacccaaaagcctttgatcagttcgaaaacgcaagctctctcgaaagaataggctgtggcgttaaaggcggcgatataaatgcgttgaggcatatgattaaaaagtcggttaccaatgataataactgtgctttttacgcctcgcggctaagtgaagagaacaaagaacgaaacgatgcgctggaacgtttactcatgggttaa

SEQ ID NO: 4 - protein, 391 aa, Serratia rubidaea
  RbwB (1)..(391)
MRVIICALGSSGDVYPCIEIGAILKERNHDVHILTNEYFKDYVESRNLSFSAVGSKEDFIRSVRDSQLWEKKTSLIKISAYMANYQVGMFHSIERLVNDNCVIIHSLWVFSAKVVSEKYSLKRFPISLTNANLKLCPGKFISWLERKLGTSLNLKAELFRRRLVSPLLQEVIASIRKSENLPADKNIYTDLVDRRLNPIILYEPWFYEKKPQHGFYMGFLLNKNRTLDHAPIINRFVDKKTVVFFTSWALSDEAGINHVLSSLKDEGLKCVLVTPTLDSIHVEENVIRTPYLNMDSIKGCLFAIHHGGIGTSAQLLKNGIPQLIYPKAFDQFENASSLERIGCGVKGGDINALRHMIKKSVTNDNNCAFYASRLSEENKERNDALERLLMG

SEQ ID NO: 5 - DNA, 888 bp, Pseudomonas aeruginosa
  rhamnosyltransferase 1, rhlA (1)..(888)
atgcggcgcgaaagtctgttggtatcggtttgcaagggcctgcgggtacatgtcgagcgcgttgggcaggatcccgggcgcagcacggtgatgctggtcaacggcgcgatggcgaccaccgcctcgttcgcccggacctgcaagtgcctggccgaacatttcaacgtggtgctgttcgacctgcccttcgccgggcagtcgcgtcagcacaacccgcagcgggggttgatcaccaaggacgacgaggtggaaatcctcctggcgctgatcgagcgcttcgaggtcaatcacctggtctccgcgtcctggggcggtatctccacgctgctggcgctgtcgcgcaatccgcgcggcatccgcagctcggtggtgatggcattcgcccctggactgaaccaggcgatgctcgactacgtcgggcgggcgcaggcgctgatcgagctggacgacaagtcggcgatcggccatctgctcaacgagaccgtcggcaaatacctgccgccgcgcctgaaagccagcaaccatcagcacatggcttcgctggccaccggcgaatacgagcaggcgcgctttcacatcgaccaggtgctggcgctcaacgatcggggctacctggcttgcctggagcggatccagagccacgtgcatttcatcaacggcagctgggacgaatacaccaccgccgaggacgcccgccagttccgcgactacctgccgcactgcagtttctcgcgggtggagggcaccgggcatttcctcgacctggagtccaagctggccgcggtacgcgtgcaccgcgccctgctcgagcacctgctgaagcaaccggagccgcagcgggcggaacgcgcggcgggattccacgagatggccatcggctacgcctga

SEQ ID NO: 6 - protein, 295 aa, Pseudomonas aeruginosa
  RhlA (1)..(295)
MRRESLLVSVCKGLRVHVERVGQDPGRSTVMLVNGAMATTASFARTCKCLAEHFNVVLFDLPFAGQSRQHNPQRGLITKDDEVEILLALIERFEVNHLVSASWGGISTLLALSRNPRGIRSSVVMAFAPGLNQAMLDYVGRAQALIELDDKSAIGHLLNETVGKYLPPRLKASNHQHMASLATGEYEQARFHIDQVLALNDRGYLACLERIQSHVHFINGSWDEYTTAEDARQFRDYLPHCSFSRVEGTGHFLDLESKLAAVRVHRALLEHLLKQPEPQRAERAAGFHEMAIGYA

SEQ ID NO: 7 - DNA, 1041 bp, Burkholderia thailandensis
atgcgcggttccggcgagtgggtagccgctgcggcgcgcgtgaggcagggcgggcagatcgcgcgggagggcggctacgtggaggcgtccatcaagggcgcgggatcagctcatttgccgagcagatgcgggagatacgccatgcctatcgagaaacaggtggtagcgctgccgagcggactgaaggtccacgtcgagcgtcatgtgttcgatccggccttcgagacggtcatcctcgtgaacggcgcgctggcgacgaccgcgtcgttcggccagacgattcgctacctgggcgaacgcgtgaacgcggtgtgcttcgacttgccgtacgcgggccagtcgcgccagcacaatccgggcgagtacattctgacgaaggacgacgaggtggagattctgctgcacctggccgagcggttcgagccgagtttcctgctgtcggtgtcgtggggcggggtggcgtcgctgttcgcgctggcgcgggggtgcgcgagcgtgcggcgggcggtgatcgcgtcgttctcgccgttcctgaacgacgcgatgacggattacgtgacgcgcgcgcgcgatcacatcgcggcgggggagaacctgaaggcggcgcagttgctcaacgacacggtggggcgctacctgccgcggatcatgaagctgtacaactaccggtatctgacgaagctgccgcgcaccgagcaggaccaggtggcgttccacgtcgaccagatcctgtcgatgcggccggagcagtacctgccggaattccgccagatcggctgcgcggtgaagttcatcaacggcgagctggacgagtacacgacggcgtcggacgtgcggcggctggcggcctacgtgcggcgcgcggagttcgcgacgatccggcaggcggggcacttcctggacctcgaggggcgtcagcagcaggagcagcttcgcgcggcgatcctgggcttcttcggcgacgagcgggcgagcgcggcgcgcgacgacgcgcaggacgagacgctcgcgccgctcggtcagttgccggcgctgtcgtag

SEQ ID NO: 8 - protein, 346 aa, Burkholderia thailandensis
MRGSGEWVAAAARVRQGGQIAREGGYVEASIKGAGSAHLPSRCGRYAMPIEKQVVALPSGLKVHVERHVFDPAFETVILVNGALATTASFGQTIRYLGERVNAVCFDLPYAGQSRQHNPGEYILTKDDEVEILLHLAERFEPSFLLSVSWGGVASLFALARGCASVRRAVIASFSPFLNDAMTDYVTRARDHIAAGENLKAAQLLNDTVGRYLPRIMKLYNYRYLTKLPRTEQDQVAFHVDQILSMRPEQYLPEFRQIGCAVKFINGELDEYTTASDVRRLAAYVRRAEFATIRQAGHFLDLEGRQQQEQLRAAILGFFGDERASAARDDAQDETLAPLGQLPALS

SEQ ID NO: 9 - DNA, 888 bp, Pseudomonas aeruginosa
atgcggcgcgaaagtctgttggtatcggtttgcaagggcctgcgggtacatgtcgagcgcgttgggcaggatcccgggcgcagcacggtgatgctggtcaacggcgcgatggcgaccaccgcctcgttcgcccggacctgcaagtgcctggccgaacatttcaacgtggtgctgttcgacctgcccttcgccgggcagtcgcgtcagcacaacccgcagcgcgggttgatcaccaaggacgacgaggtggaaatcctcctggcgctgatcgagcgcttcgaggtcaatcacctggtctccgcgtcgtggggcggtatctccacgctgctggcgctgtcgcgcaatccgcgcggcatccgcagctcggtggtgatggcattcgcccctggactgaaccaggcgatgctcgactacgtcgggcgggcgcaggcgctgatcgagctggacgacaagtcggcgatcggccatctgctcaacgagaccgtcggcaaatacctgccgccgcgcctgaaagccagcaaccatcagcacatggcttcgctggccaccggcgaatacgagcaggcgcgctttcacatcgaccaggtgctggcgctcaacgatcggggctacctggcttgcctggagcggatccagagccacgtgcatttcatcaacggcagctgggacgaatacaccaccgccgaggacgcccgccagttccgcgactacctgccgcactgcagtttctcgcgggtggagggcaccgggcatttcctcgacctggagtccaagctggccgcggtacgcgtgcaccgcgccctgctcgagcacctgctgaagcaaccggagccgcagcgggcggaacgcgcggcgggattccacgagatggccatcggctacgcctga

SEQ ID NO: 10 - protein, 295 aa, Pseudomonas aeruginosa; identical to SEQ ID NO: 6

SEQ ID NO: 11 - DNA, 888 bp, Pseudomonas aeruginosa
atgcggcgcgaaagtctgttggtatcggtttgcaagggcctgcgggtacatgtcgagcgcgttgggcaggatcccgggcgcagcacggtgatgctggtcaacggcgcgatggcgaccaccgcctcgttcgcccggacctgcaagtgcctggccgaacatttcaacgtggtgctgttcgacctgcccttcgccgggcagtcgcgtcagcacaacccgcagcgcgggttgatcaccaaggacgacgaggtggaaatcctcctggcgctgatcgagcgcttcgaggtcaatcacctggtctccgcgtcctggggcggtatctccacgctgctggcgctgtcgcgcaatccgcgcggcatccgcagctcggtggtgatggcattcgcccctggactgaaccaggcgatgctcgactacgtcgggcgggcgcaggcgctgatcgagctggacgacaagtcggcgatcggccatctgctcaacgagaccgtcggcaaatacctgccgcagcgcctgaaagccagcaaccatcagcacatggcttcgctggccaccggcgaatacgagcaggcgcgctttcacatcgaccaggtgctggcgctcaacgatcggggctacttggcttgcctggagcggatccagagccacgtgcatttcatcaacggcagctgggacgaatacaccaccgccgaggacgcccgccagttccgcgactacctgccgcactgcagtttctcgcgggtggagggcaccgggcatttcctcgacctggagtccaagctggcagcggtacgcgtgcaccgcgccctgctcgagcacctgctgaagcaaccggagccgcagcgggcggaacgcgcggcgggattccacgagatggccatcggctacgcctga

SEQ ID NO: 12 - protein, 295 aa, Pseudomonas aeruginosa
MRRESLLVSVCKGLRVHVERVGQDPGRSTVMLVNGAMATTASFARTCKCLAEHFNVVLFDLPFAGQSRQHNPQRGLITKDDEVEILLALIERFEVNHLVSASWGGISTLLALSRNPRGIRSSVVMAFAPGLNQAMLDYVGRAQALIELDDKSAIGHLLNETVGKYLPQRLKASNHQHMASLATGEYEQARFHIDQVLALNDRGYLACLERIQSHVHFINGSWDEYTTAEDARQFRDYLPHCSFSRVEGTGHFLDLESKLAAVRVHRALLEHLLKQPEPQRAERAAGFHEMAIGYA

SEQ ID NO: 13 - DNA, 888 bp, Pseudomonas aeruginosa
atgcggcgcgaaagtctgttggtaacggtatgcaagggcctgcgggtacatgtcgagcgcgtggggcaggatcccgggcgcgacacggtgatgctggtcaacggcgcgatggcgaccaccgcctcgttcgcccggacctgcaagtgcctggccgaacatttcaacgtggtgctgttcgacctgcccttcgccgggcagtcgcggcagcacaatccgcagcgcgggttgatcaccaaggacgacgaggtggagattctcctggcgctgatcgagcgcttcgctgtcaaccacctggtctcggcctcctggggcggcatctccacgctgctggcgctgtcgcgcaacccgcgcggggtccgcagctcggtggtgatggcgttcgcgccggggctgaaccaggcgatgctcgattatgtcgggcgggcccaggaactgatcgaactggacgacaagtcggcgatcggccacctgctcaacgagaccgtcggcaagtacctgccgccgcggctgaaggccagcaaccatcagcacatggcctccctggccactggcgagtacgagcaggcgcgtttccacatcgaccaggtgctggcgctcaatgaccgtggctacctgagctgcctggggcagatccagagtcacgtgcatttcatcaacggcagctgggacgagtacaccaccgccgaggacgcccgccagttccgcgattacctgccgcattgcagtttttcgcgggtggaaggcaccgggcacttcctcgacctggagtccaagctggcggcggcgcgtgtgcaccgggcgttgctcgagcacctgctggcgcaaccggaaccgtggcgctccgagcaggcggcgggattccacgagatggccatcggctacgcctga

SEQ ID NO: 14 - protein, 295 aa, Pseudomonas aeruginosa
MRRESLLVTVCKGLRVHVERVGQDPGRDTVMLVNGAMATTASFARTCKCLAEHFNVVLFDLPFAGQSRQHNPQRGLITKDDEVEILLALIERFAVNHLVSASWGGISTLLALSRNPRGVRSSVVMAFAPGLNQAMLDYVGRAQELIELDDKSAIGHLLNETVGKYLPPRLKASNHQHMASLATGEYEQARFHIDQVLALNDRGYLSCLGQIQSHVHFINGSWDEYTTAEDARQFRDYLPHCSFSRVEGTGHFLDLESKLAAARVHRALLEHLLAQPEPWRSEQAAGFHEMAIGYA

SEQ ID NO: 15 - DNA, 2084 bp, Artificial Sequence
  Synthetical operon rbwAB
tcatgggggtgggaaatgaaaccagaaacagaaattgttcgcgtcggtgactggcaggtctatgtagagcgatatatttatccaggcgtcacggattccgtcatttgcgttaatggatctttttcaaccacgctggcttttcgcagctgcgtacgtaacttcaagaaccgggttaacgtcattctcttcgatctgccgttcctcggtcagtcccgtgagcataatgatttaaccaaaccgctgtcgaaaaccgatgaggttttcattctgcagagtttgattaaccattatgaaccgtcttatctgctctccatctcctggggcggactggcagcattgatggcgctctcctcccgccctcgctccatccgcaaagccgtggtggcctcgttctccaccaaggtgaacgacgcgatgaattactacgtcagtcagggcaagaaattactggatgaaggcaaaggcgatgaagcggcgatgctgctcaataccgaggttggcaaatatctgccgaatctgttgaagcaggtgaactacgaacacttgagacagtttgacgaatcagcgcaaaaacaggtgcgttaccacgtcgcgcaaattaccgaatttaatcaggcggactatatcgataccttccggcaaatcgatacgccgatactgttcatcaacggcgagcaggacgaatacactacagcgcaagatattaaggaactcagtaactatatcaataactgcgaatttattaccgtaccgcaggctggccactttatttatatggaaagccgctttgcggccgattatttcaacgacgtgatgaacggttttctgtttgttgaagaagcgatggcctcctgaggataacaaactaaaatattgattcgacaagacaggatggtgatatgagagtgataatatgcgccctggggtcctctggcgatgtttacccatgcatcgaaattggcgcgatattaaaagaaagaaaccatgatgtgcatatacttaccaatgaatacttcaaagattacgttgagtctcgcaatctttccttttcagcagtaggcagtaaagaggactttatccgttcagtacgtgacagccagctatgggagaagaaaacctcattaataaaaatatctgcatacatggctaattatcaggttggtatgtttcattcaatcgagaggttggtaaatgataattgtgtaattattcattctctttgggtattctcagccaaggtggttagcgaaaaatattcgttaaaacgattcccgataagccttaccaacgccaaccttaaactctgcccggggaaatttattagctggttggaaagaaagctcggcacctcattgaacctgaaggctgaactctttagacgccgcctggtttctccgctgttacaggaggtcatcgcctcgataagaaaatcagagaacctcccagccgataaaaacatctataccgacctggtagataggcgcttgaatcctattattttgtatgagccttggttctacgaaaaaaaaccgcagcacggattttatatggggttcctgttaaataaaaaccggacattagaccacgctccgataatcaaccgctttgtggacaaaaaaacggtggttttcttcaccagttgggcattgtctgatgaagcaggcataaatcatgtcttaagcagtctgaaagatgaaggtttgaaatgtgtactggtcacccccaccctcgacagcatccacgttgaagaaaatgtcatcagaacaccttaccttaatatggatagcatcaaaggatgtctgtttgccattcaccacggcggcatcggcaccagtgcccaactgcttaaaaacggcatacctcagttaatctacccaaaagcctttgatcagttcgaaaacgcaagctctctcgaaagaataggctgtggcgttaaaggcggcgatataaatgcgttgaggcatatgattaaaaagtcggttaccaatgataataactgtgctttttacgcctcgcggctaagtgaagagaacaaagaacgaaacgatgcgctggaacgtttactcatgggttaagctcgagca

SEQ ID NO: 16 - DNA, 2028 bp, Artificial Sequence
  Promoter cassette Prha
ttaatctttctgcgaattgagatgacgccactggctgggcgtcatcccggtttcccgggtaaacaccaccgaaaaatagttactatcttcaaagccacattcggtcgaaatatcactgattaacaggcggctatgctggagaagatattgcgcatgacacactctgacctgtcgcagatattgattgatggtcattccagtctgctggcgaaattgctgacgcaaaacgcgctcactgcacgatgcctcatcacaaaatttatccagcgcaaagggacttttcaggctagccgccagccgggtaatcagcttatccagcaacgtttcgctggatgttggcggcaacgaatcactggtgtaacgatggcgattcagcaacatcaccaactgcccgaacagcaactcagccatttcgttagcaaacggcacatgctgactactttcatgctcaagctgaccgataacctgccgcgcctgcgccatccccatgctacctaagcgccagtgtggttgccctgcgctggcgttaaatcccggaatcgccccctgccagtcaagattcagcttcagacgctccgggcaataaataatattctgcaaaaccagatcgttaacggaagcgtaggagtgtttatcgtcagcatgaatgtaaaagagatcgccacgggtaatgcgataagggcgatcgttgagtacatgcaggccattaccgcgccagacaatcaccagctcacaaaaatcatgtgtatgttcagcaaagacatcttgcggataacggtcagccacagcgactgcctgctggtcgctggcaaaaaaatcatctttgagaagttttaactgatgcgccaccgtggctacctcggccagagaacgaagttgattattcgcaatatggcgtacaaatacgttgagaagattcgcgttattgcagaaagccatcccgtccctggcgaatatcacgcggtgaccagttaaactctcggcgaaaaagcgtcgaaaagtggttactgtcgctgaatccacagcgataggcgatgtcagtaacgctggcctcgctgtggcgtagcagatgtcgggctttcatcagtcgcaggcggttcaggtatcgctgaggcgtcagtcccgtttgctgcttaagctgccgatgtagcgtacgcagtgaaagagaaaattgatccgccacggcatcccaattcacctcatcggcaaaatggtcctccagccaggccagaagcaagttgagacgtgatgcgctgttttccaggttctcctgcaaactgcttttacgcagcaagagcagtaattgcataaacaagatctcgcgactggcggtcgagggtaaatcattttccccttcctgctgttccatctgtgcaaccagctgtcgcacctgctgcaatacgctgtggttaacgcgccagtgagacggatactgcccatccagctcttgtggcagcaactgattcagcccggcgagaaactgaaatcgatccggcgagcgatacagcacattggtcagacacagattatcggtatgttcatacagatgccgatcatgatcgcgtacgaaacagaccgtgccaccggtgatggtatagggctgcccattaaacacatgaatacccgtgccatgttcgacaatcacaatttcatgaaaatcatgatgatgttcaggaaaatccgcctgcgggagccggggttctatcgccacggacgcgttaccagacggaaaaaaatccacactatgtaatacggtcatactggcctcctgatgtcgtcaacacggcgaaatagtaatcacgaggtcaggttcttaccttaaattttcgacggaaaaccacgtaaaaaacgtcgatttttcaagatacagcgtgaattttcaggaaatgcggtgagcatcacatcaccacaattcagcaaattgtgaacatcatcacgttcatctttccctggttgccaatggcccattttcctgtcagtaacgagaaggtcgcgaattcaggcgctttttagactggtcgtaatgaa

SEQ ID NO: 17 - DNA, 107 bp, Artificial Sequence
  Terminator sequence
caaataaaacgaaaggctcagtcgaaagactgggcctttcgttttatctgttgtttgtcggtgaacgctctcctgagtaggacaaatccgccgggagcggatttgaa

SEQ ID NO: 18 - DNA, 10738 bp, Artificial Sequence
  Plasmid pACYC_rbwAB_Srub
tcaggcgggcaagaatgtgaataaaggccggataaaacttgtgcttatttttctttacggtctttaaaaaggccgtaatatccagctgaacggtctggttataggtacattgagcaactgactgaaatgcctcaaaatgttctttacgatgccattgggatatatcaacggtggtatatccagtgatttttttctccattttagcttccttagctcctgaaaatctcgataactcaaaaaatacgcccggtagtgatcttatttcattatggtgaaagttggaacctcttacgtgccgatcaacgtctcattttcgccaaaagttggcccagggcttcccggtatcaacagggacaccaggatttatttattctgcgaagtgatcttccgtcacaggtatttattcggcgcaaagtgcgtcgggtgatgctgccaacttactgatttagtgtatgatggtgtttttgaggtgctccagtggcttctgtttctatcagctgtccctcctgttcagctactgacggggtggtgcgtaacggcaaaagcaccgccggacatcagcgctagcggagtgtatactggcttactatgttggcactgatgagggtgtcagtgaagtgcttcatgtggcaggagaaaaaaggctgcaccggtgcgtcagcagaatatgtgatacaggatatattccgcttcctcgctcactgactcgctacgctcggtcgttcgactgcggcgagcggaaatggcttacgaacggggcggagatttcctggaagatgccaggaagatacttaacagggaagtgagagggccgcggcaaagccgtttttccataggctccgcccccctgacaagcatcacgaaatctgacgctcaaatcagtggtggcgaaacccgacaggactataaagataccaggcgtttccccctggcggctccctcgtgcgctctcctgttcctgcctttcggtttaccggtgtcattccgctgttatggccgcgtttgtctcattccacgcctgacactcagttccgggtaggcagttcgctccaagctggactgtatgcacgaaccccccgttcagtccgaccgctgcgccttatccggtaactatcgtcttgagtccaacccggaaagacatgcaaaagcaccactggcagcagccactggtaattgatttagaggagttagtcttgaagtcatgcgccggttaaggctaaactgaaaggacaagttttggtgactgcgctcctccaagccagttacctcggttcaaagagttggtagctcagagaaccttcgaaaaaccgccctgcaaggcggttttttcgttttcagagcaagagattacgcgcagaccaaaacgatctcaagaagatcatcttattaatcagataaaatatttctagatttcagtgcaatttatctcttcaaatgtagcacctgaagtcagccccatacgatataagttgtaattctcatgtttgacagcttatcatcgataagctttaatgcggtagtttatcacagttaaattgctaacgcagtcaggcaccgtgtatgattgaacaagatggattgcacgcaggttctccggccgcttgggtggagaggctattcggctatgactgggcacaacagacaatcggctgctctgatgccgccgtgttccggctgtcagcgcaggggcgcccggttctttttgtcaagaccgacctgtccggtgccctgaatgaactgcaggacgaggcagcgcggctatcgtggctggccacgacgggcgttccttgcgcagctgtgctcgacgttgtcactgaagcgggaagggactggctgctattgggcgaagtgccggggcaggatctcctgtcatctcaccttgctcctgccgagaaagtatccatcatggctgatgcaatgcggcggctgcatacgcttgatccggctacctgcccattcgaccaccaagcgaaacatcgcatcgagcgagcacgtactcggatggaagccggtcttgtcgatcaggatgatctggacgaagagcatcaggggctcgcgccagccgaactgttcgccaggctcaaggcgcgcatgcccgacggcgaggatctcgtcgtgacccatggcgatgcctgcttgccgaatatcatggtggaaaatggccgcttttctggattcatcgactgtggccggctgggtgtggcggaccgctatcaggacatagcgttggctacccgtgatattgctgaagagcttggcggcgaatgggctgaccgcttcctcgtgctttacggtatcgccgctcccgattcgcagcgcatcgccttctatcgccttcttgacgagttcatggaagccggcggcacctcgctaacggattcaccactccaagaattggagccaatcaattcttgcggagaactgtgaatgcgcaaaccaacccttggcagaacatatccatcgcgtccgccatctccagcagccgcacgcggcgcatctcgggcagcgttgggtcctggccacgggtgcgcatgatcgtgctcctgtcgttgaggacccggctaggctggcggggttgccttactggttagcagaatgaatcaccgatacgcgagcgaacgtgaagcgactgctgctgcaaaacgtctgcgacctgagcaacaacatgaatggtcttcggtttccgtgtttcgtaaagtctggaaacgcggaagtcccctacgtgctgctgaagttgcccgcaacagagagtggaaccaaccggtgataccacgatactatgactgagagtcaacgccatgagcggcctcatttcttattctgagttacaacagtccgcaccgctgtccggtagctccttccggtgggcgcggggcatgactatcgtcgccgcacttatgactgtcttctttatcatgcaactcgtaggacaggtgccggcagcgcccaacagtcccccggccacggggcctgccaccatacccacgccgaaacaagcgccctgcaccattatgttccggatctgcatcgcaggatgctgctggctaccctgtggaacacctacatctgtattaacgaagcgctaaccgtttttatcaggctctgggaggcagaataaatgatcatatcgtcaattattacctccacggggagagcctgagcaaactggcctcaggcatttgagaagcacacggtcacactgcttccggtagtcaataaaccggtaaaccagcaatagacataagcggctatttaacgaccctgccctgaaccgacgaccgggtcgaatttgctttcgaatttctgccattcatccgcttattatcacttattcaggcgtagcaccaggcgtttaagggcaccaataactgccttaaaaaaattacgccccgccctgccactcatcgcagtactgttgtaattcattaagcattctgccgacatggaagccatcacaaacggcatgatgaacctgaatcgccagcggcatcagcaccttgtcgccttgcgtataatatttgcccatggatttaaatttaatctttctgcgaattgagatgacgccactggctgggcgtcatcccggtttcccgggtaaacaccaccgaaaaatagttactatcttcaaagccacattcggtcgaaatatcactgattaacaggcggctatgctggagaagatattgcgcatgacacactctgacctgtcgcagatattgattgatggtcattccagtctgctggcgaaattgctgacgcaaaacgcgctcactgcacgatgcctcatcacaaaatttatccagcgcaaagggacttttcaggctagccgccagccgggtaatcagcttatccagcaacgtttcgctggatgttggcggcaacgaatcactggtgtaacgatggcgattcagcaacatcaccaactgcccgaacagcaactcagccatttcgttagcaaacggcacatgctgactactttcatgctcaagctgaccgataacctgccgcgcctgcgccatccccatgctacctaagcgccagtgtggttgccctgcgctggcgttaaatcccggaatcgccccctgccagtcaagattcagcttcagacgctccgggcaataaataatattctgcaaaaccagatcgttaacggaagcgtaggagtgtttatcgtcagcatgaatgtaaaagagatcgccacgggtaatgcgataagggcgatcgttgagtacatgcaggccattaccgcgccagacaatcaccagctcacaaaaatcatgtgtatgttcagcaaagacatcttgcggataacggtcagccacagcgactgcctgctggtcgctggcaaaaaaatcatctttgagaagttttaactgatgcgccaccgtggctacctcggccagagaacgaagttgattattcgcaatatggcgtacaaatacgttgagaagattcgcgttattgcagaaagccatcccgtccctggcgaatatcacgcggtgaccagttaaactctcggcgaaaaagcgtcgaaaagtggttactgtcgctgaatccacagcgataggcgatgtcagtaacgctggcctcgctgtggcgtagcagatgtcgggctttcatcagtcgcaggcggttcaggtatcgctgaggcgtcagtcccgtttgctgcttaagctgccgatgtagcgtacgcagtgaaagagaaaattgatccgccacggcatcccaattcacctcatcggcaaaatggtcctccagccaggccagaagcaagttgagacgtgatgcgctgttttccaggttctcctgcaaactgcttttacgcagcaagagcagtaattgcataaacaagatctcgcgactggcggtcgagggtaaatcattttccccttcctgctgttccatctgtgcaaccagctgtcgcacctgctgcaatacgctgtggttaacgcgccagtgagacggatactgcccatccagctcttgtggcagcaactgattcagcccggcgagaaactgaaatcgatccggcgagcgatacagcacattggtcagacacagattatcggtatgttcatacagatgccgatcatgatcgcgtacgaaacagaccgtgccaccggtgatggtatagggctgcccattaaacacatgaatacccgtgccatgttcgacaatcacaatttcatgaaaatcatgatgatgttcaggaaaatccgcctgcgggagccggggttctatcgccacggacgcgttaccagacggaaaaaaatccacactatgtaatacggtcatactggcctcctgatgtcgtcaacacggcgaaatagtaatcacgaggtcaggttcttaccttaaattttcgacggaaaaccacgtaaaaaacgtcgatttttcaagatacagcgtgaattttcaggaaatgcggtgagcatcacatcaccacaattcagcaaattgtgaacatcatcacgttcatctttccctggttgccaatggcccattttcctgtcagtaacgagaaggtcgcgaattcaggcgctttttagactggtcgtaatgaacatttaaatgaattcccttgggactctagagatccgcgggggcccggcatcattttattgttattcatgggggtgggaaatgaaaccagaaacagaaattgttcgcgtcggtgactggcaggtctatgtagagcgatatatttatccaggcgtcacggattccgtcatttgcgttaatggatctttttcaaccacgctggcttttcgcagctgcgtacgtaacttcaagaaccgggttaacgtcattctcttcgatctgccgttcctcggtcagtcccgtgagcataatgatttaaccaaaccgctgtcgaaaaccgatgaggttttcattctgcagagtttgattaaccattatgaaccgtcttatctgctctccatctcctggggcggactggcagcattgatggcgctctcctcccgccctcgctccatccgcaaagccgtggtggcctcgttctccaccaaggtgaacgacgcgatgaattactacgtcagtcagggcaagaaattactggatgaaggcaaaggcgatgaagcggcgatgctgctcaataccgaggttggcaaatatctgccgaatctgttgaagcaggtgaactacgaacacttgagacagtttgacgaatcagcgcaaaaacaggtgcgttaccacgtcgcgcaaattaccgaatttaatcaggcggactatatcgataccttccggcaaatcgatacgccgatactgttcatcaacggcgagcaggacgaatacactacagcgcaagatattaaggaactcagtaactatatcaataactgcgaatttattaccgtaccgcaggctggccactttatttatatggaaagccgctttgcggccgattatttcaacgacgtgatgaacggttttctgtttgttgaagaagcgatggcctcctgaggataacaaactaaaatattgattcgacaagacaggatggtgatatgagagtgataatatgcgccctggggtcctctggcgatgtttacccatgcatcgaaattggcgcgatattaaaagaaagaaaccatgatgtgcatatacttaccaatgaatacttcaaagattacgttgagtctcgcaatctttccttttcagcagtaggcagtaaagaggactttatccgttcagtacgtgacagccagctatgggagaagaaaacctcattaataaaaatatctgcatacatggctaattatcaggttggtatgtttcattcaatcgagaggttggtaaatgataattgtgtaattattcattctctttgggtattctcagccaaggtggttagcgaaaaatattcgttaaaacgattcccgataagccttaccaacgccaaccttaaactctgcccggggaaatttattagctggttggaaagaaagctcggcacctcattgaacctgaaggctgaactctttagacgccgcctggtttctccgctgttacaggaggtcatcgcctcgataagaaaatcagagaacctcccagccgataaaaacatctataccgacctggtagataggcgcttgaatcctattattttgtatgagccttggttctacgaaaaaaaaccgcagcacggattttatatggggttcctgttaaataaaaaccggacattagaccacgctccgataatcaaccgctttgtggacaaaaaaacggtggttttcttcaccagttgggcattgtctgatgaagcaggcataaatcatgtcttaagcagtctgaaagatgaaggtttgaaatgtgtactggtcacccccaccctcgacagcatccacgttgaagaaaatgtcatcagaacaccttaccttaatatggatagcatcaaaggatgtctgtttgccattcaccacggcggcatcggcaccagtgcccaactgcttaaaaacggcatacctcagttaatctacccaaaagcctttgatcagttcgaaaacgcaagctctctcgaaagaataggctgtggcgttaaaggcggcgatataaatgcgttgaggcatatgattaaaaagtcggttaccaatgataataactgtgctttttacgcctcgcggctaagtgaagagaacaaagaacgaaacgatgcgctggaacgtttactcatgggttaagctcgagcacgcgagagtagggaactgccaggcatcaaataaaacgaaaggctcagtcgaaagactgggcctttcgttttatctgttgtttgtcggtgaacgctctcctgagtaggacaaatccgccgggagcggatttgaacgatgataagctgtcaaacatgagaattcttgaagacgaaagggcctcgtgtgtacaaacgttcgtcaaaagggcgacacaaaattcctgcaggggccggcccagcgccggcggtcgagtggcgacggcgcggcttgtccgcgccctggtagattgcctggccgtaggccagccatttttgagcggccagcggccgcgataggccgacgcgaagcggcggggcgtagggagcgcagcgaccgaagggtaggcgctttttgcagctcttcggctgtgcgctggccagacagttatgcacaggccaggcgggttttaagagttttaataagttttaaagagttttaggcggaaaaatcgccttttttctcttttatatcagtcacttacatgtgtgaccggttcccaatgtacggctttgggttcccaatgtacgggttccggttcccaatgtacggctttgggttcccaatgtacgtgctatccacaggaaagagaccttttcgacctttttcccctgctagggcaatttgccctagcatctgctccgtacattaggaaccggcggatgcttcgccctcgatcaggttgcggtagcgcatgactaggatcgggccagcctgccccgcctcctccttcaaatcgtactccggcaggtcatttgacccgatcagcttgcgcacggtgaaacagaacttcttgaactctccggcgctgccactgcgttcgtagatcgtcttgaacaaccatctggcttctgccttgcctgcggcgcggcgtgccaggcggtagagaaaacggccgatgccgggatcgatcaaaaagtaatcggggtgaaccgtcagcacgtccgggttcttgccttctgtgatctcgcggtacatccaatcaactagctcgatctcgatgtactccggccgcccggtttcgctctttacgatcttgtagcggctaatcaaggcttcaccctcggataccgtcaccaggcggccgttcttggccttcttcgtacgctgcatggcaacgtgcgtggtgtttaaccgaatgcaggtttctaccaggtcgtctttctgctttccgccatcggctcgccggcagaacttgagtacgtccgcaacgtgtggacggaacacgcggccgggcttgtctcccttcccttcccggtatcggttcatggattcggttagatgggaaaccgccatcagtaccaggtcgtaatcccacacactggccatgccggccggccctgcggaaacctctacgtgcccgtctggaagctcgtagcggatcacctcgccagctcgtcggtcacgcttcgacagacggaaaacggccacgtccatgatgctgcgactatcgcgggtgcccacgtcatagagcatcggaacgaaaaaatctggttgctcgtcgcccttgggcggcttcctaatcgacggcgcaccggctgccggcggttgccgggattctttgcggattcgatcagcggccgcttgccacgattcaccggggcgtgcttctgcctcgatgcgttgccgctgggcggcctgcgcggccttcaacttctccaccaggtcatcacccagcgccgcgccgatttgtaccgggccggatggtttgcgaccgctcacgccgattcctcgggcttgggggttccagtgccattgcagggccggcagacaacccagccgcttacgcctggccaaccgcccgttcctccacacatggggcattccacggcgtcggtgcctggttgttcttgattttccatgccgcctcctttagccgctaaaattcatctactcatttattcatttgctcatttactctggtagctgcgcgatgtattcagatagcagctcggtaatggtcttgccttggcgtaccgcgtacatcttcagcttggtgtgatcctccgccggcaactgaaagttgacccgcttcatggctggcgtgtctgccaggctggccaacgttgcagccttgctgctgcgtgcgctcggacggccggcacttagcgtgtttgtgcttttgctcattttctctttacctcattaactcaaatgagttttgatttaatttcagcggccagcgcctggacctcgcgggcagcgtcgccctcgggttctgattcaagaacggttgtgccggcggcggcagtgcctgggtagctcacgcgctgcgtgatacgggactcaagaatgggcagctcgtacccggccagcgcctcggcaacctcaccgccgatgcgcgtgcctttgatcgcccgcgacacgacaaaggccgcttgtagccttccatccgtgacctcaatgcgctgcttaaccagctccaccaggtcggcggtggcccatatgtcgtaagggcttggctgcaccggaatcagcacgaagtcggctgccttgatcgcggacacagccaagtccgccgcctggggcgctccgtcgatcactacgaagtcgcgccggccgatggccttcacgtcgcggtcaatcgtcgggcggtcgatgccgacaacggttagcggttgatcttcccgcacggccgcccaatcgcgggcactgccctggggatcggaatcgactaacagaacatcggccccggcgagttgcagggcgcgggctagatgggttgcgatggtcgtcttgcctgacccgcctttctggttaagtacagcgataaccttcatgcgttccccttgcgtatttgtttatttactcatcgcatcatatacgcagcgaccgcatgacgcaagctgttttactcaaatacacatcacctttttagacggcggcgctcggtttcttcagcggccaagctggccggccaggccgccagcttggcatcagacaaaccggccaggatttcatgcagccgcacggttccggatgagcattca

SEQ ID NO: 19 - DNA, 9608 bp, Artificial Sequence
  Plasmid pACYC_rbwA_Srub
tcaggcgggcaagaatgtgaataaaggccggataaaacttgtgcttatttttctttacggtctttaaaaaggccgtaatatccagctgaacggtctggttataggtacattgagcaactgactgaaatgcctcaaaatgttctttacgatgccattgggatatatcaacggtggtatatccagtgatttttttctccattttagcttccttagctcctgaaaatctcgataactcaaaaaatacgcccggtagtgatcttatttcattatggtgaaagttggaacctcttacgtgccgatcaacgtctcattttcgccaaaagttggcccagggcttcccggtatcaacagggacaccaggatttatttattctgcgaagtgatcttccgtcacaggtatttattcggcgcaaagtgcgtcgggtgatgctgccaacttactgatttagtgtatgatggtgtttttgaggtgctccagtggcttctgtttctatcagctgtccctcctgttcagctactgacggggtggtgcgtaacggcaaaagcaccgccggacatcagcgctagcggagtgtatactggcttactatgttggcactgatgagggtgtcagtgaagtgcttcatgtggcaggagaaaaaaggctgcaccggtgcgtcagcagaatatgtgatacaggatatattccgcttcctcgctcactgactcgctacgctcggtcgttcgactgcggcgagcggaaatggcttacgaacggggcggagatttcctggaagatgccaggaagatacttaacagggaagtgagagggccgcggcaaagccgtttttccataggctccgcccccctgacaagcatcacgaaatctgacgctcaaatcagtggtggcgaaacccgacaggactataaagataccaggcgtttccccctggcggctccctcgtgcgctctcctgttcctgcctttcggtttaccggtgtcattccgctgttatggccgcgtttgtctcattccacgcctgacactcagttccgggtaggcagttcgctccaagctggactgtatgcacgaaccccccgttcagtccgaccgctgcgccttatccggtaactatcgtcttgagtccaacccggaaagacatgcaaaagcaccactggcagcagccactggtaattgatttagaggagttagtcttgaagtcatgcgccggttaaggctaaactgaaaggacaagttttggtgactgcgctcctccaagccagttacctcggttcaaagagttggtagctcagagaaccttcgaaaaaccgccctgcaaggcggttttttcgttttcagagcaagagattacgcgcagaccaaaacgatctcaagaagatcatcttattaatcagataaaatatttctagatttcagtgcaatttatctcttcaaatgtagcacctgaagtcagccccatacgatataagttgtaattctcatgtttgacagcttatcatcgataagctttaatgcggtagtttatcacagttaaattgctaacgcagtcaggcaccgtgtatgattgaacaagatggattgcacgcaggttctccggccgcttgggtggagaggctattcggctatgactgggcacaacagacaatcggctgctctgatgccgccgtgttccggctgtcagcgcaggggcgcccggttctttttgtcaagaccgacctgtccggtgccctgaatgaactgcaggacgaggcagcgcggctatcgtggctggccacgacgggcgttccttgcgcagctgtgctcgacgttgtcactgaagcgggaagggactggctgctattgggcgaagtgccggggcaggatctcctgtcatctcaccttgctcctgccgagaaagtatccatcatggctgatgcaatgcggcggctgcatacgcttgatccggctacctgcccattcgaccaccaagcgaaacatcgcatcgagcgagcacgtactcggatggaagccggtcttgtcgatcaggatgatctggacgaagagcatcaggggctcgcgccagccgaactgttcgccaggctcaaggcgcgcatgcccgacggcgaggatctcgtcgtgacccatggcgatgcctgcttgccgaatatcatggtggaaaatggccgcttttctggattcatcgactgtggccggctgggtgtggcggaccgctatcaggacatagcgttggctacccgtgatattgctgaagagcttggcggcgaatgggctgaccgcttcctcgtgctttacggtatcgccgctcccgattcgcagcgcatcgccttctatcgccttcttgacgagttcatggaagccggcggcacctcgctaacggattcaccactccaagaattggagccaatcaattcttgcggagaactgtgaatgcgcaaaccaacccttggcagaacatatccatcgcgtccgccatctccagcagccgcacgcggcgcatctcgggcagcgttgggtcctggccacgggtgcgcatgatcgtgctcctgtcgttgaggacccggctaggctggcggggttgccttactggttagcagaatgaatcaccgatacgcgagcgaacgtgaagcgactgctgctgcaaaacgtctgcgacctgagcaacaacatgaatggtcttcggtttccgtgtttcgtaaagtctggaaacgcggaagtcccctacgtgctgctgaagttgcccgcaacagagagtggaaccaaccggtgataccacgatactatgactgagagtcaacgccatgagcggcctcatttcttattctgagttacaacagtccgcaccgctgtccggtagctccttccggtgggcgcggggcatgactatcgtcgccgcacttatgactgtcttctttatcatgcaactcgtaggacaggtgccggcagcgcccaacagtcccccggccacggggcctgccaccatacccacgccgaaacaagcgccctgcaccattatgttccggatctgcatcgcaggatgctgctggctaccctgtggaacacctacatctgtattaacgaagcgctaaccgtttttatcaggctctgggaggcagaataaatgatcatatcgtcaattattacctccacggggagagcctgagcaaactggcctcaggcatttgagaagcacacggtcacactgcttccggtagtcaataaaccggtaaaccagcaatagacataagcggctatttaacgaccctgccctgaaccgacgaccgggtcgaatttgctttcgaatttctgccattcatccgcttattatcacttattcaggcgtagcaccaggcgtttaagggcaccaataactgccttaaaaaaattacgccccgccctgccactcatcgcagtactgttgtaattcattaagcattctgccgacatggaagccatcacaaacggcatgatgaacctgaatcgccagcggcatcagcaccttgtcgccttgcgtataatatttgcccatggatttaaatttaatctttctgcgaattgagatgacgccactggctgggcgtcatcccggtttcccgggtaaacaccaccgaaaaatagttactatcttcaaagccacattcggtcgaaatatcactgattaacaggcggctatgctggagaagatattgcgcatgacacactctgacctgtcgcagatattgattgatggtcattccagtctgctggcgaaattgctgacgcaaaacgcgctcactgcacgatgcctcatcacaaaatttatccagcgcaaagggacttttcaggctagccgccagccgggtaatcagcttatccagcaacgtttcgctggatgttggcggcaacgaatcactggtgtaacgatggcgattcagcaacatcaccaactgcccgaacagcaactcagccatttcgttagcaaacggcacatgctgactactttcatgctcaagctgaccgataacctgccgcgcctgcgccatccccatgctacctaagcgccagtgtggttgccctgcgctggcgttaaatcccggaatcgccccctgccagtcaagattcagcttcagacgctccgggcaataaataatattctgcaaaaccagatcgttaacggaagcgtaggagtgtttatcgtcagcatgaatgtaaaagagatcgccacgggtaatgcgataagggcgatcgttgagtacatgcaggccattaccgcgccagacaatcaccagctcacaaaaatcatgtgtatgttcagcaaagacatcttgcggataacggtcagccacagcgactgcctgctggtcgctggcaaaaaaatcatctttgagaagttttaactgatgcgccaccgtggctacctcggccagagaacgaagttgattattcgcaatatggcgtacaaatacgttgagaagattcgcgttattgcagaaagccatcccgtccctggcgaatatcacgcggtgaccagttaaactctcggcgaaaaagcgtcgaaaagtggttactgtcgctgaatccacagcgataggcgatgtcagtaacgctggcctcgctgtggcgtagcagatgtcgggctttcatcagtcgcaggcggttcaggtatcgctgaggcgtcagtcccgtttgctgcttaagctgccgatgtagcgtacgcagtgaaagagaaaattgatccgccacggcatcccaattcacctcatcggcaaaatggtcctccagccaggccagaagcaagttgagacgtgatgcgctgttttccaggttctcctgcaaactgcttttacgcagcaagagcagtaattgcataaacaagatctcgcgactggcggtcgagggtaaatcattttccccttcctgctgttccatctgtgcaaccagctgtcgcacctgctgcaatacgctgtggttaacgcgccagtgagacggatactgcccatccagctcttgtggcagcaactgattcagcccggcgagaaactgaaatcgatccggcgagcgatacagcacattggtcagacacagattatcggtatgttcatacagatgccgatcatgatcgcgtacgaaacagaccgtgccaccggtgatggtatagggctgcccattaaacacatgaatacccgtgccatgttcgacaatcacaatttcatgaaaatcatgatgatgttcaggaaaatccgcctgcgggagccggggttctatcgccacggacgcgttaccagacggaaaaaaatccacactatgtaatacggtcatactggcctcctgatgtcgtcaacacggcgaaatagtaatcacgaggtcaggttcttaccttaaattttcgacggaaaaccacgtaaaaaacgtcgatttttcaagatacagcgtgaattttcaggaaatgcggtgagcatcacatcaccacaattcagcaaattgtgaacatcatcacgttcatctttccctggttgccaatggcccattttcctgtcagtaacgagaaggtcgcgaattcaggcgctttttagactggtcgtaatgaacatttaaatgaattcccttgggactctagagatccgcgggggcccggcatcattttattgttattcatgggggtgggaaatgaaaccagaaacagaaattgttcgcgtcggtgactggcaggtctatgtagagcgatatatttatccaggcgtcacggattccgtcatttgcgttaatggatctttttcaaccacgctggcttttcgcagctgcgtacgtaacttcaagaaccgggttaacgtcattctcttcgatctgccgttcctcggtcagtcccgtgagcataatgatttaaccaaaccgctgtcgaaaaccgatgaggttttcattctgcagagtttgattaaccattatgaaccgtcttatctgctctccatctcctggggcggactggcagcattgatggcgctctcctcccgccctcgctccatccgcaaagccgtggtggcctcgttctccaccaaggtgaacgacgcgatgaattactacgtcagtcagggcaagaaattactggatgaaggcaaaggcgatgaagcggcgatgctgctcaataccgaggttggcaaatatctgccgaatctgttgaagcaggtgaactacgaacacttgagacagtttgacgaatcagcgcaaaaacaggtgcgttaccacgtcgcgcaaattaccgaatttaatcaggcggactatatcgataccttccggcaaatcgatacgccgatactgttcatcaacggcgagcaggacgaatacactacagcgcaagatattaaggaactcagtaactatatcaataactgcgaatttattaccgtaccgcaggctggccactttatttatatggaaagccgctttgcggccgattatttcaacgacgtgatgaacggttttctgtttgttgaagaagcgatggcctcctgaggataacaaactaaaatattgattcgacaagacaggatggtgatatgagagtgataatatgcgccctggggtcctctggcgatgtttacccatcgagcacgcgagagtagggaactgccaggcatcaaataaaacgaaaggctcagtcgaaagactgggcctttcgttttatctgttgtttgtcggtgaacgctctcctgagtaggacaaatccgccgggagcggatttgaacgatgataagctgtcaaacatgagaattcttgaagacgaaagggcctcgtgtgtacaaacgttcgtcaaaagggcgacacaaaattcctgcaggggccggcccagcgccggcggtcgagtggcgacggcgcggcttgtccgcgccctggtagattgcctggccgtaggccagccatttttgagcggccagcggccgcgataggccgacgcgaagcggcggggcgtagggagcgcagcgaccgaagggtaggcgctttttgcagctcttcggctgtgcgctggccagacagttatgcacaggccaggcgggttttaagagttttaataagttttaaagagttttaggcggaaaaatcgccttttttctcttttatatcagtcacttacatgtgtgaccggttcccaatgtacggctttgggttcccaatgtacgggttccggttcccaatgtacggctttgggttcccaatgtacgtgctatccacaggaaagagaccttttcgacctttttcccctgctagggcaatttgccctagcatctgctccgtacattaggaaccggcggatgcttcgccctcgatcaggttgcggtagcgcatgactaggatcgggccagcctgccccgcctcctccttcaaatcgtactccggcaggtcatttgacccgatcagcttgcgcacggtgaaacagaacttcttgaactctccggcgctgccactgcgttcgtagatcgtcttgaacaaccatctggcttctgccttgcctgcggcgcggcgtgccaggcggtagagaaaacggccgatgccgggatcgatcaaaaagtaatcggggtgaaccgtcagcacgtccgggttcttgccttctgtgatctcgcggtacatccaatcaactagctcgatctcgatgtactccggccgcccggtttcgctctttacgatcttgtagcggctaatcaaggcttcaccctcggataccgtcaccaggcggccgttcttggccttcttcgtacgctgcatggcaacgtgcgtggtgtttaaccgaatgcaggtttctaccaggtcgtctttctgctttccgccatcggctcgccggcagaacttgagtacgtccgcaacgtgtggacggaacacgcggccgggcttgtctcccttcccttcccggtatcggttcatggattcggttagatgggaaaccgccatcagtaccaggtcgtaatcccacacactggccatgccggccggccctgcggaaacctctacgtgcccgtctggaagctcgtagcggatcacctcgccagctcgtcggtcacgcttcgacagacggaaaacggccacgtccatgatgctgcgactatcgcgggtgcccacgtcatagagcatcggaacgaaaaaatctggttgctcgtcgcccttgggcggcttcctaatcgacggcgcaccggctgccggcggttgccgggattctttgcggattcgatcagcggccgcttgccacgattcaccggggcgtgcttctgcctcgatgcgttgccgctgggcggcctgcgcggccttcaacttctccaccaggtcatcacccagcgccgcgccgatttgtaccgggccggatggtttgcgaccgctcacgccgattcctcgggcttgggggttccagtgccattgcagggccggcagacaacccagccgcttacgcctggccaaccgcccgttcctccacacatggggcattccacggcgtcggtgcctggttgttcttgattttccatgccgcctcctttagccgctaaaattcatctactcatttattcatttgctcatttactctggtagctgcgcgatgtattcagatagcagctcggtaatggtcttgccttggcgtaccgcgtacatcttcagcttggtgtgatcctccgccggcaactgaaagttgacccgcttcatggctggcgtgtctgccaggctggccaacgttgcagccttgctgctgcgtgcgctcggacggccggcacttagcgtgtttgtgcttttgctcattttctctttacctcattaactcaaatgagttttgatttaatttcagcggccagcgcctggacctcgcgggcagcgtcgccctcgggttctgattcaagaacggttgtgccggcggcggcagtgcctgggtagctcacgcgctgcgtgatacgggactcaagaatgggcagctcgtacccggccagcgcctcggcaacctcaccgccgatgcgcgtgcctttgatcgcccgcgacacgacaaaggccgcttgtagccttccatccgtgacctcaatgcgctgcttaaccagctccaccaggtcggcggtggcccatatgtcgtaagggcttggctgcaccggaatcagcacgaagtcggctgccttgatcgcggacacagccaagtccgccgcctggggcgctccgtcgatcactacgaagtcgcgccggccgatggccttcacgtcgcggtcaatcgtcgggcggtcgatgccgacaacggttagcggttgatcttcccgcacggccgcccaatcgcgggcactgccctggggatcggaatcgactaacagaacatcggccccggcgagttgcagggcgcgggctagatgggttgcgatggtcgtcttgcctgacccgcctttctggttaagtacagcgataaccttcatgcgttccccttgcgtatttgtttatttactcatcgcatcatatacgcagcgaccgcatgacgcaagctgttttactcaaatacacatcacctttttagacggcggcgctcggtttcttcagcggccaagctggccggccaggccgccagcttggcatcagacaaaccggccaggatttcatgcagccgcacggttccggatgagcattca

SEQ ID NO: 20 - DNA, 2132 bp, Artificial Sequence
  Synthetical operon rhlA_Pa rbwB_Srub
tttgggaggtgtgaaatgcggcgcgaaagtctgttggtatcggtttgcaagggcctgcgggtacatgtcgagcgcgttgggcaggatcccgggcgcagcacggtgatgctggtcaacggcgcgatggcgaccaccgcctcgttcgcccggacctgcaagtgcctggccgaacatttcaacgtggtgctgttcgacctgcccttcgccgggcagtcgcgtcagcacaacccgcagcgggggttgatcaccaaggacgacgaggtggaaatcctcctggcgctgatcgagcgcttcgaggtcaatcacctggtctccgcgtcctggggcggtatctccacgctgctggcgctgtcgcgcaatccgcgcggcatccgcagctcggtggtgatggcattcgcccctggactgaaccaggcgatgctcgactacgtcgggcgggcgcaggcgctgatcgagctggacgacaagtcggcgatcggccatctgctcaacgagaccgtcggcaaatacctgccgccgcgcctgaaagccagcaaccatcagcacatggcttcgctggccaccggcgaatacgagcaggcgcgctttcacatcgaccaggtgctggcgctcaacgatcggggctacctggcttgcctggagcggatccagagccacgtgcatttcatcaacggcagctgggacgaatacaccaccgccgaggacgcccgccagttccgcgactacctgccgcactgcagtttctcgcgggtggagggcaccgggcatttcctcgacctggagtccaagctggccgcggtacgcgtgcaccgcgccctgctcgagcacctgctgaagcaaccggagccgcagcgggcggaacgcgcggcgggattccacgagatggccatcggctacgcctgaggataacaaactaaaatattgattcgacaagacaggatggtgatatgagagtgataatatgcgccctggggtcctctggcgatgtttacccatgcatcgaaattggcgcgatattaaaagaaagaaaccatgatgtgcatatacttaccaatgaatacttcaaagattacgttgagtctcgcaatctttccttttcagcagtaggcagtaaagaggactttatccgttcagtacgtgacagccagctatgggagaagaaaacctcattaataaaaatatctgcatacatggctaattatcaggttggtatgtttcattcaatcgagaggttggtaaatgataattgtgtaattattcattctctttgggtattctcagccaaggtggttagcgaaaaatattcgttaaaacgattcccgataagccttaccaacgccaaccttaaactctgcccggggaaatttattagctggttggaaagaaagctcggcacctcattgaacctgaaggctgaactctttagacgccgcctggtttctccgctgttacaggaggtcatcgcctcgataagaaaatcagagaacctcccagccgataaaaacatctataccgacctggtagataggcgcttgaatcctattattttgtatgagccttggttctacgaaaaaaaaccgcagcacggattttatatggggttcctgttaaataaaaaccggacattagaccacgctccgataatcaaccgctttgtggacaaaaaaacggtggttttcttcaccagttgggcattgtctgatgaagcaggcataaatcatgtcttaagcagtctgaaagatgaaggtttgaaatgtgtactggtcacccccaccctcgacagcatccacgttgaagaaaatgtcatcagaacaccttaccttaatatggatagcatcaaaggatgtctgtttgccattcaccacggcggcatcggcaccagtgcccaactgcttaaaaacggcatacctcagttaatctacccaaaagcctttgatcagttcgaaaacgcaagctctctcgaaagaataggctgtggcgttaaaggcggcgatataaatgcgttgaggcatatgattaaaaagtcggttaccaatgataataactgtgctttttacgcctcgcggctaagtgaagagaacaaagaacgaaacgatgcgctggaacgtttactcatgggttaagctcgagca

SEQ ID NO: 21 - DNA, 10787 bp, Artificial Sequence
  Plasmid pACYC_rhlA_Pa rbwB_Srub
tcaggcgggcaagaatgtgaataaaggccggataaaacttgtgcttatttttctttacggtctttaaaaaggccgtaatatccagctgaacggtctggttataggtacattgagcaactgactgaaatgcctcaaaatgttctttacgatgccattgggatatatcaacggtggtatatccagtgatttttttctccattttagcttccttagctcctgaaaatctcgataactcaaaaaatacgcccggtagtgatcttatttcattatggtgaaagttggaacctcttacgtgccgatcaacgtctcattttcgccaaaagttggcccagggcttcccggtatcaacagggacaccaggatttatttattctgcgaagtgatcttccgtcacaggtatttattcggcgcaaagtgcgtcgggtgatgctgccaacttactgatttagtgtatgatggtgtttttgaggtgctccagtggcttctgtttctatcagctgtccctcctgttcagctactgacggggtggtgcgtaacggcaaaagcaccgccggacatcagcgctagcggagtgtatactggcttactatgttggcactgatgagggtgtcagtgaagtgcttcatgtggcaggagaaaaaaggctgcaccggtgcgtcagcagaatatgtgatacaggatatattccgcttcctcgctcactgactcgctacgctcggtcgttcgactgcggcgagcggaaatggcttacgaacggggcggagatttcctggaagatgccaggaagatacttaacagggaagtgagagggccgcggcaaagccgtttttccataggctccgcccccctgacaagcatcacgaaatctgacgctcaaatcagtggtggcgaaacccgacaggactataaagataccaggcgtttccccctggcggctccctcgtgcgctctcctgttcctgcctttcggtttaccggtgtcattccgctgttatggccgcgtttgtctcattccacgcctgacactcagttccgggtaggcagttcgctccaagctggactgtatgcacgaaccccccgttcagtccgaccgctgcgccttatccggtaactatcgtcttgagtccaacccggaaagacatgcaaaagcaccactggcagcagccactggtaattgatttagaggagttagtcttgaagtcatgcgccggttaaggctaaactgaaaggacaagttttggtgactgcgctcctccaagccagttacctcggttcaaagagttggtagctcagagaaccttcgaaaaaccgccctgcaaggcggttttttcgttttcagagcaagagattacgcgcagaccaaaacgatctcaagaagatcatcttattaatcagataaaatatttctagatttcagtgcaatttatctcttcaaatgtagcacctgaagtcagccccatacgatataagttgtaattctcatgtttgacagcttatcatcgataagctttaatgcggtagtttatcacagttaaattgctaacgcagtcaggcaccgtgtatgattgaacaagatggattgcacgcaggttctccggccgcttgggtggagaggctattcggctatgactgggcacaacagacaatcggctgctctgatgccgccgtgttccggctgtcagcgcaggggcgcccggttctttttgtcaagaccgacctgtccggtgccctgaatgaactgcaggacgaggcagcgcggctatcgtggctggccacgacgggcgttccttgcgcagctgtgctcgacgttgtcactgaagcgggaagggactggctgctattgggcgaagtgccggggcaggatctcctgtcatctcaccttgctcctgccgagaaagtatccatcatggctgatgcaatgcggcggctgcatacgcttgatccggctacctgcccattcgaccaccaagcgaaacatcgcatcgagcgagcacgtactcggatggaagccggtcttgtcgatcaggatgatctggacgaagagcatcaggggctcgcgccagccgaactgttcgccaggctcaaggcgcgcatgcccgacggcgaggatctcgtcgtgacccatggcgatgcctgcttgccgaatatcatggtggaaaatggccgcttttctggattcatcgactgtggccggctgggtgtggcggaccgctatcaggacatagcgttggctacccgtgatattgctgaagagcttggcggcgaatgggctgaccgcttcctcgtgctttacggtatcgccgctcccgattcgcagcgcatcgccttctatcgccttcttgacgagttcatggaagccggcggcacctcgctaacggattcaccactccaagaattggagccaatcaattcttgcggagaactgtgaatgcgcaaaccaacccttggcagaacatatccatcgcgtccgccatctccagcagccgcacgcggcgcatctcgggcagcgttgggtcctggccacgggtgcgcatgatcgtgctcctgtcgttgaggacccggctaggctggcggggttgccttactggttagcagaatgaatcaccgatacgcgagcgaacgtgaagcgactgctgctgcaaaacgtctgcgacctgagcaacaacatgaatggtcttcggtttccgtgtttcgtaaagtctggaaacgcggaagtcccctacgtgctgctgaagttgcccgcaacagagagtggaaccaaccggtgataccacgatactatgactgagagtcaacgccatgagcggcctcatttcttattctgagttacaacagtccgcaccgctgtccggtagctccttccggtgggcgcggggcatgactatcgtcgccgcacttatgactgtcttctttatcatgcaactcgtaggacaggtgccggcagcgcccaacagtcccccggccacggggcctgccaccatacccacgccgaaacaagcgccctgcaccattatgttccggatctgcatcgcaggatgctgctggctaccctgtggaacacctacatctgtattaacgaagcgctaaccgtttttatcaggctctgggaggcagaataaatgatcatatcgtcaattattacctccacggggagagcctgagcaaactggcctcaggcatttgagaagcacacggtcacactgcttccggtagtcaataaaccggtaaaccagcaatagacataagcggctatttaacgaccctgccctgaaccgacgaccgggtcgaatttgctttcgaatttctgccattcatccgcttattatcacttattcaggcgtagcaccaggcgtttaagggcaccaataactgccttaaaaaaattacgccccgccctgccactcatcgcagtactgttgtaattcattaagcattctgccgacatggaagccatcacaaacggcatgatgaacctgaatcgccagcggcatcagcaccttgtcgccttgcgtataatatttgcccatggatttaaatttaatctttctgcgaattgagatgacgccactggctgggcgtcatcccggtttcccgggtaaacaccaccgaaaaatagttactatcttcaaagccacattcggtcgaaatatcactgattaacaggcggctatgctggagaagatattgcgcatgacacactctgacctgtcgcagatattgattgatggtcattccagtctgctggcgaaattgctgacgcaaaacgcgctcactgcacgatgcctcatcacaaaatttatccagcgcaaagggacttttcaggctagccgccagccgggtaatcagcttatccagcaacgtttcgctggatgttggcggcaacgaatcactggtgtaacgatggcgattcagcaacatcaccaactgcccgaacagcaactcagccatttcgttagcaaacggcacatgctgactactttcatgctcaagctgaccgataacctgccgcgcctgcgccatccccatgctacctaagcgccagtgtggttgccctgcgctggcgttaaatcccggaatcgccccctgccagtcaagattcagcttcagacgctccgggcaataaataatattctgcaaaaccagatcgttaacggaagcgtaggagtgtttatcgtcagcatgaatgtaaaagagatcgccacgggtaatgcgataagggcgatcgttgagtacatgcaggccattaccgcgccagacaatcaccagctcacaaaaatcatgtgtatgttcagcaaagacatcttgcggataacggtcagccacagcgactgcctgctggtcgctggcaaaaaaatcatctttgagaagttttaactgatgcgccaccgtggctacctcggccagagaacgaagttgattattcgcaatatggcgtacaaatacgttgagaagattcgcgttattgcagaaagccatcccgtccctggcgaatatcacgcggtgaccagttaaactctcggcgaaaaagcgtcgaaaagtggttactgtcgctgaatccacagcgataggcgatgtcagtaacgctggcctcgctgtggcgtagcagatgtcgggctttcatcagtcgcaggcggttcaggtatcgctgaggcgtcagtcccgtttgctgcttaagctgccgatgtagcgtacgcagtgaaagagaaaattgatccgccacggcatcccaattcacctcatcggcaaaatggtcctccagccaggccagaagcaagttgagacgtgatgcgctgttttccaggttctcctgcaaactgcttttacgcagcaagagcagtaattgcataaacaagatctcgcgactggcggtcgagggtaaatcattttccccttcctgctgttccatctgtgcaaccagctgtcgcacctgctgcaatacgctgtggttaacgcgccagtgagacggatactgcccatccagctcttgtggcagcaactgattcagcccggcgagaaactgaaatcgatccggcgagcgatacagcacattggtcagacacagattatcggtatgttcatacagatgccgatcatgatcgcgtacgaaacagaccgtgccaccggtgatggtatagggctgcccattaaacacatgaatacccgtgccatgttcgacaatcacaatttcatgaaaatcatgatgatgttcaggaaaatccgcctgcgggagccggggttctatcgccacggacgcgttaccagacggaaaaaaatccacactatgtaatacggtcatactggcctcctgatgtcgtcaacacggcgaaatagtaatcacgaggtcaggttcttaccttaaattttcgacggaaaaccacgtaaaaaacgtcgatttttcaagatacagcgtgaattttcaggaaatgcggtgagcatcacatcaccacaattcagcaaattgtgaacatcatcacgttcatctttccctggttgccaatggcccattttcctgtcagtaacgagaaggtcgcgaattcaggcgctttttagactggtcgtaatgaacatttaaatgaattcccttgggactctagagatccgcgggggcccaggaggggggatctggcatttttgggaggtgtgaaatgcggcgcgaaagtctgttggtatcggtttgcaagggcctgcgggtacatgtcgagcgcgttgggcaggatcccgggcgcagcacggtgatgctggtcaacggcgcgatggcgaccaccgcctcgttcgcccggacctgcaagtgcctggccgaacatttcaacgtggtgctgttcgacctgcccttcgccgggcagtcgcgtcagcacaacccgcagcgggggttgatcaccaaggacgacgaggtggaaatcctcctggcgctgatcgagcgcttcgaggtcaatcacctggtctccgcgtcctggggcggtatctccacgctgctggcgctgtcgcgcaatccgcgcggcatccgcagctcggtggtgatggcattcgcccctggactgaaccaggcgatgctcgactacgtcgggcgggcgcaggcgctgatcgagctggacgacaagtcggcgatcggccatctgctcaacgagaccgtcggcaaatacctgccgccgcgcctgaaagccagcaaccatcagcacatggcttcgctggccaccggcgaatacgagcaggcgcgctttcacatcgaccaggtgctggcgctcaacgatcggggctacctggcttgcctggagcggatccagagccacgtgcatttcatcaacggcagctgggacgaatacaccaccgccgaggacgcccgccagttccgcgactacctgccgcactgcagtttctcgcgggtggagggcaccgggcatttcctcgacctggagtccaagctggccgcggtacgcgtgcaccgcgccctgctcgagcacctgctgaagcaaccggagccgcagcgggcggaacgcgcggcgggattccacgagatggccatcggctacgcctgaggataacaaactaaaatattgattcgacaagacaggatggtgatatgagagtgataatatgcgccctggggtcctctggcgatgtttacccatgcatcgaaattggcgcgatattaaaagaaagaaaccatgatgtgcatatacttaccaatgaatacttcaaagattacgttgagtctcgcaatctttccttttcagcagtaggcagtaaagaggactttatccgttcagtacgtgacagccagctatgggagaagaaaacctcattaataaaaatatctgcatacatggctaattatcaggttggtatgtttcattcaatcgagaggttggtaaatgataattgtgtaattattcattctctttgggtattctcagccaaggtggttagcgaaaaatattcgttaaaacgattcccgataagccttaccaacgccaaccttaaactctgcccggggaaatttattagctggttggaaagaaagctcggcacctcattgaacctgaaggctgaactctttagacgccgcctggtttctccgctgttacaggaggtcatcgcctcgataagaaaatcagagaacctcccagccgataaaaacatctataccgacctggtagataggcgcttgaatcctattattttgtatgagccttggttctacgaaaaaaaaccgcagcacggattttatatggggttcctgttaaataaaaaccggacattagaccacgctccgataatcaaccgctttgtggacaaaaaaacggtggttttcttcaccagttgggcattgtctgatgaagcaggcataaatcatgtcttaagcagtctgaaagatgaaggtttgaaatgtgtactggtcacccccaccctcgacagcatccacgttgaagaaaatgtcatcagaacaccttaccttaatatggatagcatcaaaggatgtctgtttgccattcaccacggcggcatcggcaccagtgcccaactgcttaaaaacggcatacctcagttaatctacccaaaagcctttgatcagttcgaaaacgcaagctctctcgaaagaataggctgtggcgttaaaggcggcgatataaatgcgttgaggcatatgattaaaaagtcggttaccaatgataataactgtgctttttacgcctcgcggctaagtgaagagaacaaagaacgaaacgatgcgctggaacgtttactcatgggttaagctcgagcacgcgagagtagggaactgccaggcatcaaataaaacgaaaggctcagtcgaaagactgggcctttcgttttatctgttgtttgtcggtgaacgctctcctgagtaggacaaatccgccgggagcggatttgaacgatgataagctgtcaaacatgagaattcttgaagacgaaagggcctcgtgtgtacaaacgttcgtcaaaagggcgacacaaaattcctgcaggggccggcccagcgccggcggtcgagtggcgacggcgcggcttgtccgcgccctggtagattgcctggccgtaggccagccatttttgagcggccagcggccgcgataggccgacgcgaagcggcggggcgtagggagcgcagcgaccgaagggtaggcgctttttgcagctcttcggctgtgcgctggccagacagttatgcacaggccaggcgggttttaagagttttaataagttttaaagagttttaggcggaaaaatcgccttttttctcttttatatcagtcacttacatgtgtgaccggttcccaatgtacggctttgggttcccaatgtacgggttccggttcccaatgtacggctttgggttcccaatgtacgtgctatccacaggaaagagaccttttcgacctttttcccctgctagggcaatttgccctagcatctgctccgtacattaggaaccggcggatgcttcgccctcgatcaggttgcggtagcgcatgactaggatcgggccagcctgccccgcctcctccttcaaatcgtactccggcaggtcatttgacccgatcagcttgcgcacggtgaaacagaacttcttgaactctccggcgctgccactgcgttcgtagatcgtcttgaacaaccatctggcttctgccttgcctgcggcgcggcgtgccaggcggtagagaaaacggccgatgccgggatcgatcaaaaagtaatcggggtgaaccgtcagcacgtccgggttcttgccttctgtgatctcgcggtacatccaatcaactagctcgatctcgatgtactccggccgcccggtttcgctctttacgatcttgtagcggctaatcaaggcttcaccctcggataccgtcaccaggcggccgttcttggccttcttcgtacgctgcatggcaacgtgcgtggtgtttaaccgaatgcaggtttctaccaggtcgtctttctgctttccgccatcggctcgccggcagaacttgagtacgtccgcaacgtgtggacggaacacgcggccgggcttgtctcccttcccttcccggtatcggttcatggattcggttagatgggaaaccgccatcagtaccaggtcgtaatcccacacactggccatgccggccggccctgcggaaacctctacgtgcccgtctggaagctcgtagcggatcacctcgccagctcgtcggtcacgcttcgacagacggaaaacggccacgtccatgatgctgcgactatcgcgggtgcccacgtcatagagcatcggaacgaaaaaatctggttgctcgtcgcccttgggcggcttcctaatcgacggcgcaccggctgccggcggttgccgggattctttgcggattcgatcagcggccgcttgccacgattcaccggggcgtgcttctgcctcgatgcgttgccgctgggcggcctgcgcggccttcaacttctccaccaggtcatcacccagcgccgcgccgatttgtaccgggccggatggtttgcgaccgctcacgccgattcctcgggcttgggggttccagtgccattgcagggccggcagacaacccagccgcttacgcctggccaaccgcccgttcctccacacatggggcattccacggcgtcggtgcctggttgttcttgattttccatgccgcctcctttagccgctaaaattcatctactcatttattcatttgctcatttactctggtagctgcgcgatgtattcagatagcagctcggtaatggtcttgccttggcgtaccgcgtacatcttcagcttggtgtgatcctccgccggcaactgaaagttgacccgcttcatggctggcgtgtctgccaggctggccaacgttgcagccttgctgctgcgtgcgctcggacggccggcacttagcgtgtttgtgcttttgctcattttctctttacctcattaactcaaatgagttttgatttaatttcagcggccagcgcctggacctcgcgggcagcgtcgccctcgggttctgattcaagaacggttgtgccggcggcggcagtgcctgggtagctcacgcgctgcgtgatacgggactcaagaatgggcagctcgtacccggccagcgcctcggcaacctcaccgccgatgcgcgtgcctttgatcgcccgcgacacgacaaaggccgcttgtagccttccatccgtgacctcaatgcgctgcttaaccagctccaccaggtcggcggtggcccatatgtcgtaagggcttggctgcaccggaatcagcacgaagtcggctgccttgatcgcggacacagccaagtccgccgcctggggcgctccgtcgatcactacgaagtcgcgccggccgatggccttcacgtcgcggtcaatcgtcgggcggtcgatgccgacaacggttagcggttgatcttcccgcacggccgcccaatcgcgggcactgccctggggatcggaatcgactaacagaacatcggccccggcgagttgcagggcgcgggctagatgggttgcgatggtcgtcttgcctgacccgcctttctggttaagtacagcgataaccttcatgcgttccccttgcgtatttgtttatttactcatcgcatcatatacgcagcgaccgcatgacgcaagctgttttactcaaatacacatcacctttttagacggcggcgctcggtttcttcagcggccaagctggccggccaggccgccagcttggcatcagacaaaccggccaggatttcatgcagccgcacggttccggatgagcattca